European Patent Application EP 4 155 412 A1, published March 29, 2023. Title: Method for determining formulation of combination of plurality of candidates for smell or taste for reproducing smell or taste of target substance. Applicant: Japan Tobacco Inc. The sequence listing filed with the application follows.

SEQUENCE LISTING (7 sequences)

SEQ ID NO: 1 - DNA, 1146 bp, Homo sapiens
  CDS (1)..(1146)
atggggtgtttgggcggcaacagcaagacgacggaagaccagggcgtcgatgaaaaagaacgacgcgaggccaacaaaaagatcgagaagcagttgcagaaagagcgcctggcttacaaggctacccaccgcctgctgctcctgggggctggtgagtctgggaaaagcactatcgtcaaacagatgaggatcctgcacgtcaatgggtttaatcccgaggaaaagaaacagaaaattctggacatccggaaaaatgttaaagatgctatcgtgacaattgtttcagcaatgagtactataatacctccagttccgctggccaaccctgaaaaccaatttcgatcagactacatcaagagcatagcccctatcactgactttgaatattcccaggaattctttgaccatgtgaaaaaactttgggacgatgaaggcgtgaaggcatgctttgagagatccaacgaataccagctgattgactgtgcacaatacttcctggaaagaatcgacagcgtcagcttggttgactacacacccacagaccaggacctcctcagatgcagagttctgacatctgggatttttgagacacgattccaagtggacaaagtaaacttccacatgtttgatgttggtggccagagggatgagaggagaaaatggatccagtgctttaacgatgtcacagctatcatttacgtcgcagcctgcagtagctacaacatggtgattcgagaagataacaacaccaacaggctgagagagtccctggatctttttgaaagcatctggaacaacaggtggttacggaccatttctatcatcttgttcttgaacaaacaagatatgctggcagaaaaagtcttggcagggaaatcaaaaattgaagactatttcccagaatatgcaaattatactgttcctgaagacgcaacaccagatgcaggagaagatcccaaagttacaagagccaagttctttatccgggacctgtttttgaggatcagcacggccaccggtgacggcaaacattactgctacccgcacttcacctgcgccgtggacacagagaacatccgcagggtgttcaacgactgccgcgacatcatccagcggatgcacctcaagcagtatgagctcttgtga

SEQ ID NO: 2 - protein, 381 aa, Homo sapiens
MGCLGGNSKTTEDQGVDEKERREANKKIEKQLQKERLAYKATHRLLLLGAGESGKSTIVKQMRILHVNGFNPEEKKQKILDIRKNVKDAIVTIVSAMSTIIPPVPLANPENQFRSDYIKSIAPITDFEYSQEFFDHVKKLWDDEGVKACFERSNEYQLIDCAQYFLERIDSVSLVDYTPTDQDLLRCRVLTSGIFETRFQVDKVNFHMFDVGGQRDERRKWIQCFNDVTAIIYVAACSSYNMVIREDNNTNRLRESLDLFESIWNNRWLRTISIILFLNKQDMLAEKVLAGKSKIEDYFPEYANYTVPEDATPDAGEDPKVTRAKFFIRDLFLRISTATGDGKHYCYPHFTCAVDTENIRRVFNDCRDIIQRMHLKQYELL

SEQ ID NO: 3 - DNA, 684 bp, Homo sapiens
  CDS (1)..(684)
atgtgtaaaagcgtgaccacagatgagtggaagaaagtcttctatgagaagatggaggaggcaaagccggctgacagctgggacctcatcatagaccccaacctcaagcacaatgtgctgagccctggttggaagcagtacctggaattgcatgcttcaggcaggttccactgctcctggtgctggcacacctggcagtcgccctacgtggtcatcctcttccacatgttcctggaccgcgcccagcgggcgggctcggtgcgcatgcgcgtcttcaagcagctgtgctatgagtgcggcacggcgcggctggacgagtccagcatgctggaggagaacatcgagggcctggtggacaacctcatcaccagcctgcgcgagcagtgctacggcgagcgtggcggccagtaccgcatccacgtggccagccgccaggacaaccggcggcaccgcggagagttctgcgaggcctgccaggagggcatcgtgcactggaagcccagcgagaagctgctggaggaggaggcgaccacctacaccttctcccgggcgcccagccccaccaagtcgcaggaccagacgggctcaggctggaacttctgctctatcccctggtgcttgttttgggccacggtcctgctgctgatcatctacctgcagttctctttccgtagctccgtataa

SEQ ID NO: 4 - protein, 227 aa, Homo sapiens
MCKSVTTDEWKKVFYEKMEEAKPADSWDLIIDPNLKHNVLSPGWKQYLELHASGRFHCSWCWHTWQSPYVVILFHMFLDRAQRAGSVRMRVFKQLCYECGTARLDESSMLEENIEGLVDNLITSLREQCYGERGGQYRIHVASRQDNRRHRGEFCEACQEGIVHWKPSEKLLEEEATTYTFSRAPSPTKSQDQTGSGWNFCSIPWCLFWATVLLLIIYLQFSFRSSV

SEQ ID NO: 5 - DNA, 672 bp, Mus musculus
  CDS (1)..(672)
atgtccaccagcctgaccacttgtgagtggaagaaggtcttctacgagaagatggaggtggccaagccagcggacagctgggagctcatcatagaccccaccctcaagcccaatgagctgggccctggctggaagcagtacctggagcaacatgcctcaggcaggttccactgttcctggtgttggcacacatggcaatctgccaatgtcgtcattctcttccacatgcacctggaccgtgcccagcgtgttggctcagtgcgcatgcgcgtgttcaagcagctgtgctatcagtgcggcacgtcgcggctggacgagtccagcatgctggaggagaatatcgagggcctggtggacaacctcatcaccagtctgcgcgagcagtgttacgatgaggatggtggccagtaccgcatccacgtagccagccggccagacagcggattgcaccgcagtgagttctgcgaggcctgccaggaaggcatcgtgcactggaagcccagcgaaaagctgctggaggaggatgccgcctataccgatgcctccaagaagaagggccaggctggttttatctccagcttcttctcatttcgttggtgcctgttctggggcaccctctgcctggtcattgtctacctgcagttcttccgaggccgctctggcttcctttag

SEQ ID NO: 6 - protein, 223 aa, Mus musculus
MSTSLTTCEWKKVFYEKMEVAKPADSWELIIDPTLKPNELGPGWKQYLEQHASGRFHCSWCWHTWQSANVVILFHMHLDRAQRVGSVRMRVFKQLCYQCGTSRLDESSMLEENIEGLVDNLITSLREQCYDEDGGQYRIHVASRPDSGLHRSEFCEACQEGIVHWKPSEKLLEEDAAYTDASKKKGQAGFISSFFSFRWCLFWGTLCLVIVYLQFFRGRSGFL

SEQ ID NO: 7 - DNA, 63 bp, picornavirus
ggaagcggagagggcaggggaagtcttctaacatgcggggacgtggaggaaaatcccggcccc